European Patent Application EP 4 190 146 A1, published June 7, 2023. Title: Brassica oleracea plants with improved nutritional value. Applicant: Seminis Vegetable Seeds, Inc. The sequence listing filed with the application follows.

SEQUENCE LISTING (9 sequences)

SEQ ID NO: 1 - DNA, 20 bp, synthetic construct
  misc_feature 1..20: note = Primer
  source 1..20: mol_type = other DNA
cggattttcaaattttctcg

SEQ ID NO: 2 - DNA, 20 bp, synthetic construct
  misc_feature 1..20: note = Primer
  source 1..20: mol_type = other DNA
atttcgcatgaccactaggc

SEQ ID NO: 3 - DNA, 196 bp, synthetic construct
  misc_feature 1..196: note = Taqman assay NBOLI009111370
  source 1..196: mol_type = other DNA
gaccacctaaagacaagaatagtgaaagagataagatggaagaccaaagttaatcaaatttattttgaagcttttytatggaatagagactaaaatgatgtgtgctattgcaatttttagtcacatattgctaatcaaacacatattttgcatcagagaattgtcaaatacatgaaaaaaataaagaataattttt

SEQ ID NO: 4 - DNA, 29 bp, synthetic construct
  misc_feature 1..29: note = Forward primer
  source 1..29: mol_type = other DNA
gtgaaagagataagatggaagaccaaagt

SEQ ID NO: 5 - DNA, 29 bp, synthetic construct
  misc_feature 1..29: note = Reverse primer
  source 1..29: mol_type = other DNA
gtgactaaaaattgcaatagcacacatca

SEQ ID NO: 6 - DNA, 17 bp, synthetic construct
  misc_feature 1..17: note = Vic probe
  source 1..17: mol_type = other DNA
ctattccatagaaaagc

SEQ ID NO: 7 - DNA, 17 bp, synthetic construct
  misc_feature 1..17: note = Fam probe
  source 1..17: mol_type = other DNA
ctattccataaaaaagc

SEQ ID NO: 8 - DNA, 2165 bp, Brassica villosa FT69
  source 1..2165: mol_type = genomic DNA
gaaaatcacagttcacgcctcttactccatgagcttctctattctcatcctagtgttataatcttgcaaacacatatagaaagcaagatttggagtgtacgagaaaaacatgaaaacacctagaagctctgtgggtaagacccaagagcgtttctcgattagtttcatatacagatgcatcagagttctcatcaaccgatctacttctttcttatcttattagaaaaaaaaaatcctatcaaaatttactttcctgcaagtatatttttctttacattttcattttcttgagtgttatttgagtgaagttatattaaaatattgttcatatatatcgaaaatgtcaagaaagccatgttgtgtcggagaagggctgaagaaaggggcatggaccaccgaggaagataagaaactcatctcttacatccatgaacatggagaaggaggctggcgcgacattcctcaaaaagctggttaatatctattatatattttttggtaaatttttaaaacatatatgtttgtttggtatttgatgtatgaaagttttatattgaatgtggtgttttactaggattgaaaaggtgtggaaagagttgcagactgcgatggactaactacctaaaacctgagatcaaaagaggcgagtttagttcagaggaggaacagattatcatcatgctccatgctgctcgtggcaacaagtacgtttattttagaccaaaaaaaaacaagtacgtttatttttaacaaaaaggacgattatatatttttgtgtgtatggatcctccagtgatcatcattctagttttctcttcttttttttataccgcaaacaaatttcattagtaaaaaaaattaaaattccaaagtcaatattcaaaaacacagtgttatataatcctatatatgtcatatattaaaaaagtatattaaaaaagtacaacatgagaaatgaatttaagtatgcttctaaagcgaagttttacttcccaaaaaattattctttatttttttcatgtatttgacaattctctgatgcaaaatatgtgtttgattagcaatatgtgactaaaaattgcaatagcacacatcattttagtctctattccatagaaaagcttcaaaataaatttgattaactttggtcttccatcttatctctttcactattcttgtctttaggtggtcggtcatagckagacatttacctagaagaacmgacaatgagatcaagaaytactggaacacacatctcaagaaacgtttgatcgaacagggtactgatcccgtgactcacaagccactagcttctaatacaaaccctactgtacctgagaatttgcattccctagatgcatctagttccgacaagcaatactcccggtcaagctcaatgccttccatgtcttgtactccttcctccggtttcaacacggttttcgagaataccagcaaagatgggacaccagttcgtgaggacgattccttgagtcgcaagaaacgtttgaagaaatcaagttctacatcaaggcttttgaacaaagttgcggctaaggccacttccatgaaaaaagctttgtctgcttccatggaaggtagcttgaatgctaatataagcttttccaatggctactctgagcagattctcaatgaagatgatagttctaatgcatccctcataaacactctcgccgagttcgatcccttcctccaaacaacgttttaccctgagaatgagatgaatactacttctgatctcggtatagatcaggactacttctcacattttctcgaaaatttcggcaaccataatgaggagcactacatgaatcataactatggtcatggtcttcttatgtcctatgtgtcccaagaagtctcatcaactagcgttgatgatcaagacaatactaatgagggttggtcaaattatcttcttgaccatgctgattttatacatgacatggattctgattccctcggaaagcatctcatatgaatcttcgtgcctaagcagaaaggtttcaaacttgtcagaacaagaagttatgtatgtattctattatatggattgtttagtatatgtccaagatcatggttgttagtcccaagtttagggtttgtataatatacaataagggacgttatcttataaaacgagg

SEQ ID NO: 9 - DNA, 2186 bp, Brassica oleracea
  source 1..2186: mol_type = genomic DNA
gaaaatcacagttcacgcctcttactccatgagcttctctattctcatcctagtgttataatcttgcaaacacatatagaaagcaaggtttggagtgtacgagaaaaacatgaaaacacctagaagctctgtgggtgagacccaagagcgtttctcgattagtttcatatacagatgcatcagagttctcatcaaccgatctacttctttcttatcttattagaagaaaaaaatcctatcaaaatttactttcctgcaagtatatttttctttacattttcattttcttgagtgttatttgagtgaagttatattaaaatattgtaatagagttcatatatatcgaaaatgtcaagaaagccatgttgtgtcggagaagggctgaagaaaggggcatggaccaccgaggaagataagaaactcatctcttacatccatgaacatggagaaggaggctggcgcgacattcctcaaaaagctggttaatatctattatatattttttggtaaatttttaaaacatatatatgtttgtttggtatttgatgtatgaaagttttatgttgaatatggtgttttactaggrttgaaaaggtgtggaaagagttgtagactgcgatggactaactacctaaaacctgagatcaaaagaggcgagtttagttcagaggaggaacagattatcatcatgctccatgctgctcgtggcaacaagtacgtttattttagaccaaaaaaaaacaagtacgtttatttttaacaaaaaggacgattatatatttttatgtgtgtatggatcctccagtgatcatcattctagttttctctttttttttataccgcaaacaaatttcattagtaaaaaaattaaaattccaaagtcaatattcaaaaacacagtgttatatatataatcctatatatgtcatatattaaaaaagtacaacatgagaaatgaatttaagtatgcttctaaagcgaagttttacttcccgaaaaattattctttatttttttcatgtatttgacaattctctgatgcaaaatatgtgtttgattagcaatatgtgactaaaaattgcaatagcacacatcattttagtctctattccataaaaaagcttcaaaataaatttgattaactttggtcttccatcttatctctttcactattcttgtctttaggtggtcggtcatagckagacatttacctagaagaacmgacaatgagatcaagaactactggaacacacatctcaagaaacgtttgatcgaacagggtactgatcccgtgactcacaagccactagcttctaatacaaaccctactgtacctgagaatttgcattccctagatgcatctagtaattccgacaagcaatactcccggtcaagctcaatgccttccatgtcttgtactccttcctccggtttcaacacggttttcgagaataccagcaaagatgggacaccagttcgtgaggacgattccttgagtcgcaagaaacgttttaagaaatcaagttctacatcaaggcttttgaacaaagttgcggctaaggccacttccatgaaagaagctttgtctgcttccatggaaggtagtttgaatgctaatacaagcttttccaatggctactctgagcagattctcaatgaagatgatagttctaatgcatccctcataaacactctcgccgagttcgatcccttcctccaaacaacgttttaccctgagaatgagatgaatactacttctgatctcggtatagatcaggactacttctcacattttctcgaaaatttcggcagagatgatgaccacaatgaggagcactacatgaatcataactatggtcatgatcttcttatgtccgatgtgtcccaagaagtctcatcaactagcgttgatgatcaagacaatactaatgagggttggtcaaattatcttcttgaccatgctgattttatacatgacatggattctgattccctcggaaagcatctcatatgaatcttcgtgcccaagcagaaaggtttcaaacttttgaaacttgtcagaacaagaagttatgtatgtattctattatatggattgtttagtatatgtccaagatcatggttgttagtcccaagtttagggtttgtataatatacaataagggacgttatcttataaaacgagg